European Patent Specification EP 3 200 831 B1, published June 4, 2025. Title: VACCINES WITH INTERLEUKIN-21 AS AN ADJUVANT. Applicant: THE TRUSTEES OF THE UNIVERSITY OF PENNSYLVANIA Inovio Pharmaceuticals, Inc. WEINER, David MORROW, Matthew P. The sequence listing filed with the application follows.

SEQUENCE LISTING (9 sequences)

SEQ ID NO: 1 - DNA, 495 bp, Artificial Sequence
  chemically synthesized
atggactggacctggatcctgttcctggtcgccgcagccacaagggtgcacagcgagaggaccctggtctgcctggtggtgatcttcctgggcaccgtggcccacaagagcagcccccagggccccgacaggctgctgatcaggctgaggcacctgatcgacatcgtggagcagctgaagatctacgagaacgacctggaccccgagctgctctccgcccctcaagacgtgaagggccactgcgagcacgccgccttcgcctgcttccagaaggccaagctgaagcccagcaaccccggcaacaacaagaccttcatcatcgacctggtggcccagctgagaagaaggctgcccgccagaaggggcggcaagaagcagaaacacatcgccaagtgccccagctgcgacagctacgagaagaggacccccaaggaatttctggagaggctgaagtggctgctgcagaagatgattcaccagcacctgagctgatga

SEQ ID NO: 2 - protein, 163 aa, Artificial Sequence
  chemically synthesized
MDWTWILFLVAAATRVHSERTLVCLVVIFLGTVAHKSSPQGPDRLLIRLRHLIDIVEQLKIYENDLDPELLSAPQDVKGHCEHAAFACFQKAKLKPSNPGNNKTFIIDLVAQLRRRLPARRGGKKQKHIAKCPSCDSYEKRTPKEFLERLKWLLQKMIHQHLS

SEQ ID NO: 3 - DNA, 537 bp, Artificial Sequence
  chemically synthesized
atggactggacttggattctgtttctggtcgcagcagcaactagagtgcattcacgcagcagccctgggaacatggagaggattgtcatctgcctgatggtgattttcctgggcacactggtccacaagagctcctctcagggacaggacaggcatatgatcaggatgcgacagctgatcgacatcgtggatcagctgaagaactacgtgaacgacctggtcccagagtttctgcctgcaccagaggatgtcgaaactaactgcgaatggagtgccttctcatgtttccagaaggcacagctgaagtccgctaacaccggaaacaatgagcgaatcatcaacgtgagcattaagaaactgaagcgaaagccccctagtaccaatgctggccggagacagaagcacagactgacatgccctagctgtgattcctacgaaaagaaaccacccaaggagttcctggaacgctttaaaagcctgctgcagaaaatgattcaccagcacctgtcttccagaacccacggctcagaggattca

SEQ ID NO: 4 - protein, 179 aa, Artificial Sequence
  chemically synthesized
MDWTWILFLVAAATRVHSRSSPGNMERIVICLMVIFLGTLVHKSSSQGQDRHMIRMRQLIDIVDQLKNYVNDLVPEFLPAPEDVETNCEWSAFSCFQKAQLKSANTGNNERIINVSIKKLKRKPPSTNAGRRQKHRLTCPSCDSYEKKPPKEFLERFKSLLQKMIHQHLSSRTHGSEDS

SEQ ID NO: 5 - DNA, 2142 bp, Artificial Sequence
  chemically synthesized
ggatccatggactggacctggattctgttcctggtggccgccgccaccagagtgcacagcagagtgatgggcatccagcggaattgccagcacctgtggagatggggcaccatgatcctgggcatgatcatcatctgctctgccgccgagaacctgtgggtgaccgtgtactacggcgtgcctgtgtggaaggacgccgagaccaccctgttctgcgccagcgacgccaaggcctacgataccgaagtgcacaatgtgtgggccacccacgcctgcgtgcctaccgatcccaacccccaggagatcaacctggagaacgtgaccgaggagttcaacatgtggaagaacaacatggtggagcagatgcacaccgacatcatcagcctgtgggaccagagcctgaagccttgcgtgaagctgacccctctgtgcgtgaccctgaactgcagcaacgtgaacgtgaccaccaacatcatgaagggcgagatcaagaactgcagcttcaacatgaccaccgagctgcgggacaagaagcagaaagtgtacagcctgttctacaagctggacgtggtgcagatcaacaagagcaacagcagcagccagtaccggctgatcaactgcaacaccagcgccatcacccaggcctgccccaaagtgagcttcgagcccatccccatccactactgcgcccctgccggcttcgccatcctgaagtgcaaggacaaggagtttaacggcaccggcccctgcaagaatgtgagcaccgtgcagtgcacccacggcatcaagcccgtggtgtccacccagctgctgctgaacggcagcctggccgaggaggaagtgatgatccggagcgagaacatcaccaacaacgccaagaacatcatcgtgcagctgaccaagcccgtgaagatcaattgcacccggcccaacaacaacacccggaagagcatcagaatcggccctggccaggccttctacgccaccggcgacatcatcggcgatatcaggcaggcccactgcaatgtgagccggaccgagtggaacgagaccctgcagaaagtggccaagcagctgcggaagtacttcaacaacaagaccatcatcttcaccaacagcagcggcggcagactgagaatcaccacccacagcttcaattgtggcggcgagttcttctactgcaatacctccggcctgttcaacagcacctggaacggcaacggcaccaagaagaagaacagcaccgagagcaacgacaccatcaccctgccctgccggatcaagcagatcatcaatatgtggcagagggtgggccaggccatgtacgcccctcccatccagggcgtgatcagatgcgagagcaacatcaccggcctgctgctgaccagagatggcggcgacaacaacagcaagaacgagaccttcagacctggcggcggagacatgagggacaactggcggagcgagctgtacaagtacaaagtggtgaagatcgagcccctgggcgtggcccccaccaaggccaagagaagagtggtggagcgggagaagagagctgtgggcatcggcgccgtgttcctgggcttcctgggagccgccggaagcaccatgggagccgccagcatcaccctgaccgtgcaggccagacagctgctgagcggcattgtgcagcagcagagcaacctgctgagagccatcgaggcccagcagcacctgctgaagctgacagtgtggggcatcaaacagctgcaggcccgcgtgctggccgtggagagatacctgaaggaccagcagctgctgggcatctggggctgcagcggcaagctgatctgcaccaccaacgtgccctggaatagcagctggagcaacaagagccagagcgagatctgggacaacatgacctggctgcagtgggacaaggagatcagcaactacaccgatatcatctacaacctgatcgaggagagccagaaccagcaggagaagaacgagcaggatctgctggccctggacaagtgggccaacctgtggaactggttcgacatcagcaactggctgtggtacatcaagatcttcatcatgattgtgggcggcctgatcggcctgagaatcgtgttcgccgtgctgtctgtgtgactcgag

SEQ ID NO: 6 - protein, 709 aa, Artificial Sequence
  chemically synthesized
MDWTWILFLVAAATRVHSRVMGIQRNCQHLWRWGTMILGMIIICSAAENLWVTVYYGVPVWKDAETTLFCASDAKAYDTEVHNVWATHACVPTDPNPQEINLENVTEEFNMWKNNMVEQMHTDIISLWDQSLKPCVKLTPLCVTLNCSNVNVTTNIMKGEIKNCSFNMTTELRDKKQKVYSLFYKLDVVQINKSNSSSQYRLINCNTSAITQACPKVSFEPIPIHYCAPAGFAILKCKDKEFNGTGPCKNVSTVQCTHGIKPVVSTQLLLNGSLAEEEVMIRSENITNNAKNIIVQLTKPVKINCTRPNNNTRKSIRIGPGQAFYATGDIIGDIRQAHCNVSRTEWNETLQKVAKQLRKYFNNKTIIFTNSSGGRLRITTHSFNCGGEFFYCNTSGLFNSTWNGNGTKKKNSTESNDTITLPCRIKQIINMWQRVGQAMYAPPIQGVIRCESNITGLLLTRDGGDNNSKNETFRPGGGDMRDNWRSELYKYKVVKIEPLGVAPTKAKRRVVEREKRAVGIGAVFLGFLGAAGSTMGAASITLTVQARQLLSGIVQQQSNLLRAIEAQQHLLKLTVWGIKQLQARVLAVERYLKDQQLLGIWGCSGKLICTTNVPWNSSWSNKSQSEIWDNMTWLQWDKEISNYTDIIYNLIEESQNQQEKNEQDLLALDKWANLWNWFDISNWLWYIKIFIMIVGGLIGLRIVFAVLSV

SEQ ID NO: 7 - DNA, 2140 bp, Artificial Sequence
  chemically synthesized
ggatccgccaccatggattggacctggattctgttcctggtggccgccgccacaagagtgcacagcagagtgcggggcatcctgagaaattgccagcagtggtggatctggggcattctggggttctggatgctgatgatctgcaacgtgatgggcaacctgtgggtgaccgtgtactacggcgtgcctgtgtggaaggaggccaagaccaccctgttctgtgccagcgatgccaaggcctacgagaccgaggtgcacaatgtgtgggccacccacgcctgtgtgcccaccgatcccaaccctcaggagatggtgctggagaacgtgaccgagaacttcaacatgtggaagaacgacatggtggaccagatgcacgaggacatcatcagcctgtgggaccagagcctgaagccttgcgtgaagctgacccctctgtgcgtgaccctgaactgccggaacaacgtgaacaacaacaacaccatgaaggaggagatcaagaactgcagcttcaacatcaccaccgagctgcgggacaagaagcagaaggtgtacgccctgttctaccggctggacatcgtgcccctgaacgagaagaacaacagcaacgactaccggctgatcaactgcaacaccagcgccatcacccaggcctgtcccaaggtgtccttcgaccccatccccatccactattgtgcccctgccggctacgccatcctgaagtgcaacaacaagaccttcaacggcaccggcccctgcaataatgtgagcaccgtgcagtgtacccacggcatcaagcctgtggtgtccacccagctgctgctgaatggcagcctggccgaggaggagattatcatccggagcgagaacctgaccaacaacgccaagaccatcattgtgcacctgaatgagagcgtggagatcgtgtgtacccggcccaacaacaatacccggaagagcatcagaatcggccctggccagaccttttacgccaccggcgacatcatcggcgatatcaggcaggcccactgcaatatcagcgaggagaagtggaacaagaccctgcagcgggtgtccgagaagctgaaggagcacttccccaataagaccatcaagttcgcccctagcagcggcggcagactggagatcaccacccacagcttcaactgcaggggcgagttcttctactgcaataccagcaagctgttcaacagcacctacatgcccaacagcaccaacaataccaacaccaccatcaccctgccctgccggatcaagcagatcatcaatatgtggcaggaagtgggcagagccatgtacgcccctcccatcgagggcaacatcacctgcaagtccaacatcaccggcctgctgctgacaagagatggcggcaagaacgacaccaatgacaccgagaccttcagacctggcggcggagacatgagggacaactggcggagcgagctgtacaagtacaaggtggtggagatcaagcctctgggcgtggcccctaccaaggccaagaggagagtggtggagagggagaagagagccgtgggcatcggcgccgtgtttctgggctttctgggagccgccggatctacaatgggagccgccagcatcacactgaccgtgcaggccagacagctgctgagcggcatcgtgcagcagcagagcaatctgctgagagccatcgaggcccagcagcacatgctgcagctgacagtgtggggcatcaagcagctgcagaccagagtgctggccatcgagcgctacctgaaggatcagcagctgctgggcatctggggctgtagcggcaagctgatctgtaccaccgccgtgccttggaatagcagctggagcaacaagagccaggaggacatctgggacaacatgacctggatgcagtgggaccgggagatcagcaactacaccgacaccatctacaggctgctggaggacagccagaaccagcaggagaagaacgagaaggacctgctggccctggacagctggaagaacctgtggaactggttcgacatcaccaactggctgtggtacatcaagatcttcatcatgattgtgggcggcctgatcggcctgagaatcatcttcgccgtgctgagcatctgatagcggccgc

SEQ ID NO: 8 - protein, 705 aa, Artificial Sequence
  chemically synthesized
MDWTWILFLVAAATRVHSRVRGILRNCQQWWIWGILGFWMLMICNVMGNLWVTVYYGVPVWKEAKTTLFCASDAKAYETEVHNVWATHACVPTDPNPQEMVLENVTENFNMWKNDMVDQMHEDIISLWDQSLKPCVKLTPLCVTLNCRNNVNNNNTMKEEIKNCSFNITTELRDKKQKVYALFYRLDIVPLNEKNNSNDYRLINCNTSAITQACPKVSFDPIPIHYCAPAGYAILKCNNKTFNGTGPCNNVSTVQCTHGIKPVVSTQLLLNGSLAEEEIIIRSENLTNNAKTIIVHLNESVEIVCTRPNNNTRKSIRIGPGQTFYATGDIIGDIRQAHCNISEEKWNKTLQRVSEKLKEHFPNKTIKFAPSSGGRLEITTHSFNCRGEFFYCNTSKLFNSTYMPNSTNNTNTTITLPCRIKQIINMWQEVGRAMYAPPIEGNITCKSNITGLLLTRDGGKNDTNDTETFRPGGGDMRDNWRSELYKYKVVEIKPLGVAPTKAKRRVVEREKRAVGIGAVFLGFLGAAGSTMGAASITLTVQARQLLSGIVQQQSNLLRAIEAQQHMLQLTVWGIKQLQTRVLAIERYLKDQQLLGIWGCSGKLICTTAVPWNSSWSNKSQEDIWDNMTWMQWDREISNYTDTIYRLLEDSQNQQEKNEKDLLALDSWKNLWNWFDITNWLWYIKIFIMIVGGLIGLRIIFAVLSI

SEQ ID NO: 9 - protein, 9 aa, Artificial Sequence
  chemically synthesized
YPYDVPDYA